European Patent Application EP 4 470 554 A1, published December 4, 2024. Title: USE OF KALLIKREIN I OR DERIVATIVE THEREOF IN THE TREATMENT OF VCI, PSCI OR CSVD. Applicant: ZonHon Biopharma Institute, Inc. Application EP. The sequence listing filed with the application follows.

SEQUENCE LISTING (5 sequences)

SEQ ID NO: 1 - protein, 238 aa, synthetic construct
IVGGWECEQHSQPWQAALYHFSTFQCGGILVHRQWVLTAAHCISDNYQLWLGRHNLFDDENTAQFVHVSESFPHPGFNMSLLENHTRQADEDYSHDLMLLRLTEPADTITDAVKVVELPTQEPEVGSTCLASGWGSIEPEQFSFPDDLQCVDLKILPNDECKKAHVQKVTDFMLCVGHLEGGKDTCVGDSGGPLMCDGVLQGVTSWGYVPCGTPNKPSVAVRVLSYVKWIEDTIAENS

SEQ ID NO: 2 - protein, 238 aa, synthetic construct
IVGGWECEQHSQPWQAALYHFSTFQCGGILVHRQWVLTAAHCISDNYQLWLGRHNLFDDENTAQFVHVSESFPHPGFNMSLLENHTRQADEDYSHDLMLLRLTEPADTITDAVKVVELPTQEPEVGSTCLASGWGSIEPEDFSFPDDLQCVDLKILPNDECKKAHVQKVTDFMLCVGHLEGGKDTCVGDSGGPLMCDGVLQGVTSWGYVPCGTPNKPSVAVRVLSYVKWIEDTIAENS

SEQ ID NO: 3 - protein, 238 aa, synthetic construct
IVGGWECEQHSQPWQAALYHFSTFQCGGILVHRQWVLTAAHCISDNYQLWLGRHNLFDDENTAQFVHVSESFPHPGFNMSLLENHTRQADEDYSHDLMLLRLTEPADTITDAVKVVELPTQEPEVGSTCLASGWGSIEPERFSFPDDLQCVDLKILPNDECKKAHVQKVTDFMLCVGHLEGGKDTCVGDSGGPLMCDGVLQGVTSWGYVPCGTPNKPSVAVRVLSYVKWIEDTIAENS

SEQ ID NO: 4 - protein, 238 aa, synthetic construct
IVGGWECEQHSQPWQAALYHFSTFQCGGILVHRQWVLTAAHCISDNYQLWLGRHNLFDDENTAQFVHVSESFPHPGFNMSLLENHTRQADEDYSHDLMLLRLTEPADTITDAVKVVELPTQEPEVGSTCLASGWGSIEPEAFSFPDDLQCVDLKILPNDECKKAHVQKVTDFMLCVGHLEGGKDTCVGDSGGPLMCDGVLQGVTSWGYVPCGTPNKPSVAVRVLSYVKWIEDTIAENS

SEQ ID NO: 5 - protein, 238 aa, synthetic construct [sequence omitted]